European Patent Application EP 4 239 072 A1, published September 6, 2023. Title: RECOMBINANT NUCLEIC ACID MOLECULE BASED ON POINT MUTATION OF TRANSLATION INITIATION ELEMENT AND USE THEREOF IN PREPARATION OF CIRCULAR RNA. Applicant: Suzhou Curemed Biomedical Technology Co. Ltd. The sequence listing filed with the application follows.

SEQUENCE LISTING (34 sequences)

SEQ ID NO: 1 - DNA, 748 bp, synthetic construct
  misc_feature 1..748: note = sequence of IRES
  source 1..748: mol_type = other DNA
tttaaaacagctctagggttgttcccaccctagaggcccaagtggcggctagcactctggtattacggtacctttgtgcgcctgttttatatcccttcccccatgtaacttagaagatattaaacaaagttcaataggagggggtacaaaccagtgccaccacgaacaaacacttctgtttccccggtgaagctacatagactgttcccacggttgaaagtggcagatccgttatccgctttggtacttcgagaaacctagtaccaccttggaatcttcgatgcgttgcgctcagcactcaaccccagagtgtagcttaggtcgatgagtctggacgatcctcactggcgacagtggtccaggctgcgttggcggcctacctgtggcgaaagccacaggacgctagttgtgaacaaggtgtgaagagtctattgagctaccaaagagtcctccggcccctgaatgcggctaatcccaaccacggagcaagtgcccacaaaccagtgggtggcttgtcgtaatgcgtaagtctgtggcggaaccgactactttgggtgtccgtgtttccttttatttttatcatggctgcttatggtgacaatctaagattgttatcatatagctattggattggccatccggtgactaacagagatcttgcatacctgtttgttggttttactaaactagatatagttacatttaaaactcttctttatatcatacagttgaatagtagaaagagaaa

SEQ ID NO: 2 - DNA, 665 bp, synthetic construct
  misc_feature 1..665: note = sequence of IRES
  source 1..665: mol_type = other DNA
gcccgtccccctcaccctcttttccggtggccacgcccgggccaccgatacttcccttcactccctcgggactgttggggaggaacacaacagggctcccctgtatttcctcttcccattccccctttcctaaccccaaccgccgtatctggtggcggtaagacacacgggtctttccctctaaagcacaattgtgtgtgtgtcccaggtcctcctgcgttcggtgcgggagtgctcccacccaactgttgtaagcctgtccaacgtgtcgtcctggcaagactatgacgtcgcatgttccgctgtggatgccgaccgggtaaccggttccccagtgtgtgtagtgcgatcttccaggttctcctggttggcgttgtccagaaactgcttcgggtaagtggggtgtgcccaatccctacaagggttgattctttcaccaccttaggaatgctccggaggtaccccagcaacagctgggatctgaccggaggctaattgtctacgggtggtgtttccattttctttttcacacaacttcattgctgacaactcactgactaatcacttgctctcttgtgcctttctgctctggttcaagttccttgattgtttgtttgattgcttttcactgctttcttcccacaatccttgctcagttcaaagtc

SEQ ID NO: 3 - DNA, 742 bp, synthetic construct
  misc_feature 1..742: note = sequence of IRES
  source 1..742: mol_type = other DNA
ttaaaacagcctgtgggttgatcccacccacagggcccactgggcgctagcactctggtatcacggtacctttgtgcgcctgttttatacttcctcccccaactgcaacttagaagtaacacaaaccgatcaacagtcagcgtggcacaccagccacgttttgatcaaacacttctgttaccccggactgagtatcaatagactgctcacgcggttgaaggagaaaacgttcgttatccggccaactacttcgagaaacctagtaacgccatggaagttgtggagtgtttcgctcagcactaccccagtgtagatcaggttgatgagtcaccgcattccccacgggtgaccgtggcggtggctgcgttggcggcctgcccatggggaaacccatgggacgctcttatacagacatggtgcgaagagtctattgagctagttggtagtcctccggcccctgaatgcggctaatcccaactgcggagcatacactctcaagccagagggtagtgtgtcgtaatgggcaactctgcagcggaaccgactactttgggtgtccgtgtttcattttattcctatactggctgcttatggtgacaattgagagattgttaccatatagctattggattggccatccggtgactaacagagctattatatatctttttgttgggtttataccacttagcttgaaagaggttaaaactctacattacattttaatactgaacaccgcaaa

SEQ ID NO: 4 - DNA, 748 bp, synthetic construct
  misc_feature 1..748: note = sequence of edited IRES
  source 1..748: mol_type = other DNA
tttaaaacagctcttgggtctttcccaccctagaggcccaagtggcggctagcactctggtattacggtacctttgtgcgcctgttttatatcccttcccccatgtaacttagaagatattaaacaaagttcaataggagggggtacaaaccagtgccaccacgaacaaacacttctgtttccccggtgaagctacatagactgttcccacggttgaaagtggcagatccgttatccgctttggtacttcgagaaacctagtaccaccttggaatcttcgatgcgttgcgctcagcactcaaccccagagtgtagcttaggtcgatgagtctggacgatcctcactggcgacagtggtccaggctgcgttggcggcctacctgtggcgaaagccacaggacgctagttgtgaacaaggtgtgaagagtctattgagctaccaaagagtcctccggcccctgaatgcggctaatcccaaccacggagcaagtgcccacaaaccagtgggtggcttgtcgtaatgcgtaagtctgtggcggaaccgactactttgggtgtccgtgtttccttttatttttatcatggctgcttatggtgacaatctaagattgttatcatatagctattggattggccatccggtgactaacagagatcttgcatacctgtttgttggttttactaaactagatatagttacatttaaaactcttctttatatcatacagttgaatagtagaaagagaaa

SEQ ID NO: 5 - DNA, 748 bp, synthetic construct
  misc_feature 1..748: note = sequence of edited IRES
  source 1..748: mol_type = other DNA
tttaaaacagctctagggttgttcccaccctagaggcccaagtggcggctagcactctggtattacggtacctttgtgcgcctgttttatatcccttcccccatgtaacttagaagatattaaacaaagttcaataggagggggtacaaaccagtgccaccacgaacaaacacttctgtttccccggtgaagctacatagactgttcccacggttgaaagtggcagatccgttatccgctttggtacttcgagaaacctagtaccaccttggaatcttcgatgcgttgcgctcagcactcaaccccagagtgtagcttaggtcgatgagtctggacgatcctcactggcgacagtggtccaggctgcgttggcggcctacctgtggcgaaagccacaggacgctagttgtgaacaaggtgtgaagagtctattgagctaccaaagagtcctccggcccctgaatgcggctaatcccaaccacggagcaagtgcccacaaaccagtgggtggcttgtcgtaatgcgtaagtctgtggcggaaccgactactttgggtgtccgtgtttccttttatttttatcatggctgcttatggtgacaatctaagattgttatcatatagctattggattggccatccggtgactaacagagatcttgcatacctgtttgttgggtctactaaactagatatagttacatttaaaactcttctttatatcatacagttgaatagtagaaagagaaa

SEQ ID NO: 6 - DNA, 665 bp, synthetic construct
  misc_feature 1..665: note = sequence of edited IRES
  source 1..665: mol_type = other DNA
gcccgtccccctcaccctcttttccggtggccacgcccgggccaccgatacttcccttcactccctcgggactgttgggtctgaacacaacagggctcccctgtatttcctcttcccattccccctttcctaaccccaaccgccgtatctggtggcggtaagacacacgggtctttccctctaaagcacaattgtgtgtgtgtcccaggtcctcctgcgttcggtgcgggagtgctcccacccaactgttgtaagcctgtccaacgtgtcgtcctggcaagactatgacgtcgcatgttccgctgtggatgccgaccgggtaaccggttccccagtgtgtgtagtgcgatcttccaggttctcctggttggcgttgtccagaaactgcttcgggtaagtggggtgtgcccaatccctacaagggttgattctttcaccaccttaggaatgctccggaggtaccccagcaacagctgggatctgaccggaggctaattgtctacgggtggtgtttccattttctttttcacacaacttcattgctgacaactcactgactaatcacttgctctcttgtgcctttctgctctggttcaagttccttgattgtttgtttgattgcttttcactgctttcttcccacaatccttgctcagttcaaagtc

SEQ ID NO: 7 - DNA, 742 bp, synthetic construct
  misc_feature 1..742: note = sequence of edited IRES
  source 1..742: mol_type = other DNA
ttaaaacagcctttgggtctatcccacccacagggcccactgggcgctagcactctggtatcacggtacctttgtgcgcctgttttatacttcctcccccaactgcaacttagaagtaacacaaaccgatcaacagtcagcgtggcacaccagccacgttttgatcaaacacttctgttaccccggactgagtatcaatagactgctcacgcggttgaaggagaaaacgttcgttatccggccaactacttcgagaaacctagtaacgccatggaagttgtggagtgtttcgctcagcactaccccagtgtagatcaggttgatgagtcaccgcattccccacgggtgaccgtggcggtggctgcgttggcggcctgcccatggggaaacccatgggacgctcttatacagacatggtgcgaagagtctattgagctagttggtagtcctccggcccctgaatgcggctaatcccaactgcggagcatacactctcaagccagagggtagtgtgtcgtaatgggcaactctgcagcggaaccgactactttgggtgtccgtgtttcattttattcctatactggctgcttatggtgacaattgagagattgttaccatatagctattggattggccatccggtgactaacagagctattatatatctttttgttgggtttataccacttagcttgaaagaggttaaaactctacattacattttaatactgaacaccgcaaa

SEQ ID NO: 8 - DNA, 128 bp, synthetic construct
  misc_feature 1..128: note = sequence of intron region I
  source 1..128: mol_type = other DNA
taattgaggcctgagtataaggtgacttatacttgtaatctatctaaacggggaacctctctagtagacaatcccgtgctaaattgtaggactaccgtcagttgctcactgtgcatcagatttctaga

SEQ ID NO: 9 - DNA, 222 bp, synthetic construct
  misc_feature 1..222: note = sequence of intron region II
  source 1..222: mol_type = other DNA
ggatcctaatacgactcactatagggagaccctcgcacagtgagcaactgacggaggttctacataaatgcctaacgactatccctttggggagtagggtcaagtgactcgaaacgatagacaacttgctttaacaagttggagatatagtctgctctgcatggtgacatgcagctggatataattccggggtaagattaacgaccttatctgaacataatg

SEQ ID NO: 10 - DNA, 1626 bp, synthetic construct
  misc_feature 1..1626: note = sequence of coding region
  source 1..1626: mol_type = other DNA
atgtgccaccagcagctggtgatcagctggttcagcctggtgttcctggccagccccctggtggccatctgggagctgaagaaggacgtgtacgtggtggagctggactggtaccccgacgcccccggcgagatggtggtgctgacctgcgacacccccgaggaggacggcatcacctggaccctggaccagagcagcgaggtgctgggcagcggcaagaccctgaccatccaggtgaaggagttcggcgacgccggccagtacacctgccacaagggcggcgaggtgctgagccacagcctgctgctgctccacaagaaggaggacggcatctggagcaccgacatcctgaaggaccagaaggagcccaagaacaagaccttcctgaggtgcgaggccaagaactacagcggcaggttcacctgctggtggctgaccaccatcagcaccgacctgaccttcagcgtgaagagcagcaggggcagcagcgacccccagggcgtgacctgcggcgctgccacattgtctgctgaaagggttagaggcgacaacaaggagtacgaatacagcgtggagtgccaggaggacagcgcctgccccgccgccgaggagagcctgcccatcgaggtgatggtggacgccgtgcacaagctgaagtacgagaactacaccagcagcttcttcatcagggacatcatcaagcccgaccctcccaagaacctgcagctgaagcccctgaagaacagcaggcaggtggaggtgagctgggagtaccccgacacctggagcacccctcacagctacttcagcctgaccttctgcgtgcaggtccagggcaagagcaagcgggagaagaaggacagggtgttcaccgacaagaccagcgccaccgtgatctgcaggaagaacgccagcatcagcgtgagggcccaggacaggtactacagcagcagctggagcgagtgggccagcgtgccctgcagcggcagcagcggcggcgggggcagccccggcggcggcagcagcaggaacctgcccgtggccacccctgatcccggaatgttcccttgcctgcaccacagccagaacctgctgagggccgtgagcaacatgctgcagaaggccaggcagaccctggagttctacccctgcaccagcgaggagatcgaccacgaggacatcaccaaggacaagaccagcaccgtggaggcctgtctgcccttggagctgaccaagaacgagagctgcctgaacagcagggaaaccagcttcatcaccaacggcagctgcctggccagcaggaagaccagcttcatgatggccctgtgcctgagcagcatctacgaggacctgaagatgtaccaggtggagttcaagaccatgaacgccaagctgctgatggaccccaagaggcagatcttcctggaccagaacatgctggccgtgatcgacgagctgatgcaggccctgaacttcaacagcgaaaccgtgccccagaagagcagcctggaggagcccgacttctacaagaccaagatcaagctgtgcatcctgctgcacgccttcaggatcagagccgtgaccatcgacagggtgatgagctacctgaacgccagctgatgatga

SEQ ID NO: 11 - DNA, 19 bp, synthetic construct
  misc_feature 1..19: note = sequence of truncated region I from translation Initiationelement
  source 1..19: mol_type = other DNA
tttaaaacagctcttgggt

SEQ ID NO: 12 - DNA, 729 bp, synthetic construct
  misc_feature 1..729: note = sequence of truncated region II from translation Initiationelement
  source 1..729: mol_type = other DNA
ctttcccaccctagaggcccaagtggcggctagcactctggtattacggtacctttgtgcgcctgttttatatcccttcccccatgtaacttagaagatattaaacaaagttcaataggagggggtacaaaccagtgccaccacgaacaaacacttctgtttccccggtgaagctacatagactgttcccacggttgaaagtggcagatccgttatccgctttggtacttcgagaaacctagtaccaccttggaatcttcgatgcgttgcgctcagcactcaaccccagagtgtagcttaggtcgatgagtctggacgatcctcactggcgacagtggtccaggctgcgttggcggcctacctgtggcgaaagccacaggacgctagttgtgaacaaggtgtgaagagtctattgagctaccaaagagtcctccggcccctgaatgcggctaatcccaaccacggagcaagtgcccacaaaccagtgggtggcttgtcgtaatgcgtaagtctgtggcggaaccgactactttgggtgtccgtgtttccttttatttttatcatggctgcttatggtgacaatctaagattgttatcatatagctattggattggccatccggtgactaacagagatcttgcatacctgtttgttggttttactaaactagatatagttacatttaaaactcttctttatatcatacagttgaatagtagaaagagaaa

SEQ ID NO: 13 - DNA, 678 bp, synthetic construct
  misc_feature 1..678: note = sequence of truncated region I from translation Initiationelement
  source 1..678: mol_type = other DNA
tttaaaacagctctagggttgttcccaccctagaggcccaagtggcggctagcactctggtattacggtacctttgtgcgcctgttttatatcccttcccccatgtaacttagaagatattaaacaaagttcaataggagggggtacaaaccagtgccaccacgaacaaacacttctgtttccccggtgaagctacatagactgttcccacggttgaaagtggcagatccgttatccgctttggtacttcgagaaacctagtaccaccttggaatcttcgatgcgttgcgctcagcactcaaccccagagtgtagcttaggtcgatgagtctggacgatcctcactggcgacagtggtccaggctgcgttggcggcctacctgtggcgaaagccacaggacgctagttgtgaacaaggtgtgaagagtctattgagctaccaaagagtcctccggcccctgaatgcggctaatcccaaccacggagcaagtgcccacaaaccagtgggtggcttgtcgtaatgcgtaagtctgtggcggaaccgactactttgggtgtccgtgtttccttttatttttatcatggctgcttatggtgacaatctaagattgttatcatatagctattggattggccatccggtgactaacagagatcttgcatacctgtttgttgggt

SEQ ID NO: 14 - DNA, 70 bp, synthetic construct
  misc_feature 1..70: note = sequence of truncated region II from translation Initiationelement
  source 1..70: mol_type = other DNA
ctactaaactagatatagttacatttaaaactcttctttatatcatacagttgaatagtagaaagagaaa

SEQ ID NO: 15 - DNA, 80 bp, synthetic construct
  misc_feature 1..80: note = sequence of truncated region I from translation Initiationelement
  source 1..80: mol_type = other DNA
gcccgtccccctcaccctcttttccggtggccacgcccgggccaccgatacttcccttcactccctcgggactgttgggt

SEQ ID NO: 16 - DNA, 585 bp, synthetic construct
  misc_feature 1..585: note = sequence of truncated region II from translation Initiationelement
  source 1..585: mol_type = other DNA
ctgaacacaacagggctcccctgtatttcctcttcccattccccctttcctaaccccaaccgccgtatctggtggcggtaagacacacgggtctttccctctaaagcacaattgtgtgtgtgtcccaggtcctcctgcgttcggtgcgggagtgctcccacccaactgttgtaagcctgtccaacgtgtcgtcctggcaagactatgacgtcgcatgttccgctgtggatgccgaccgggtaaccggttccccagtgtgtgtagtgcgatcttccaggttctcctggttggcgttgtccagaaactgcttcgggtaagtggggtgtgcccaatccctacaagggttgattctttcaccaccttaggaatgctccggaggtaccccagcaacagctgggatctgaccggaggctaattgtctacgggtggtgtttccattttctttttcacacaacttcattgctgacaactcactgactaatcacttgctctcttgtgcctttctgctctggttcaagttccttgattgtttgtttgattgcttttcactgctttcttcccacaatccttgctcagttcaaagtc

SEQ ID NO: 17 - DNA, 18 bp, synthetic construct
  misc_feature 1..18: note = sequence of truncated region I from translation Initiationelement
  source 1..18: mol_type = other DNA
ttaaaacagcctttgggt

SEQ ID NO: 18 - DNA, 724 bp, synthetic construct
  misc_feature 1..724: note = sequence of truncated region II from translation Initiationelement
  source 1..724: mol_type = other DNA
ctatcccacccacagggcccactgggcgctagcactctggtatcacggtacctttgtgcgcctgttttatacttcctcccccaactgcaacttagaagtaacacaaaccgatcaacagtcagcgtggcacaccagccacgttttgatcaaacacttctgttaccccggactgagtatcaatagactgctcacgcggttgaaggagaaaacgttcgttatccggccaactacttcgagaaacctagtaacgccatggaagttgtggagtgtttcgctcagcactaccccagtgtagatcaggttgatgagtcaccgcattccccacgggtgaccgtggcggtggctgcgttggcggcctgcccatggggaaacccatgggacgctcttatacagacatggtgcgaagagtctattgagctagttggtagtcctccggcccctgaatgcggctaatcccaactgcggagcatacactctcaagccagagggtagtgtgtcgtaatgggcaactctgcagcggaaccgactactttgggtgtccgtgtttcattttattcctatactggctgcttatggtgacaattgagagattgttaccatatagctattggattggccatccggtgactaacagagctattatatatctttttgttgggtttataccacttagcttgaaagaggttaaaactctacattacattttaatactgaacaccgcaaa

SEQ ID NO: 19 - DNA, 163 bp, synthetic construct
  misc_feature 1..163: note = sequence of intron region II
  source 1..163: mol_type = other DNA
ctacataaatgcctaacgactatccctttggggagtagggtcaagtgactcgaaacgatagacaacttgctttaacaagttggagatatagtctgctctgcatggtgacatgcagctggatataattccggggtaagattaacgaccttatctgaacataatg

SEQ ID NO: 20 - DNA, 93 bp, synthetic construct
  misc_feature 1..93: note = sequence of intron region I
  source 1..93: mol_type = other DNA
taattgaggcctgagtataaggtgacttatacttgtaatctatctaaacggggaacctctctagtagacaatcccgtgctaaattgtaggact

SEQ ID NO: 21 - DNA, 20 bp, synthetic construct
  misc_feature 1..20: note = primer sequence
  source 1..20: mol_type = other DNA
tgggaggattctgcattacc

SEQ ID NO: 22 - DNA, 18 bp, synthetic construct
  misc_feature 1..18: note = primer sequence
  source 1..18: mol_type = other DNA
cagcatcgctggttgaga

SEQ ID NO: 23 - DNA, 20 bp, synthetic construct
  misc_feature 1..20: note = primer sequence
  source 1..20: mol_type = other DNA
ctcccggcacagaagtgtat

SEQ ID NO: 24 - DNA, 20 bp, synthetic construct
  misc_feature 1..20: note = primer sequence
  source 1..20: mol_type = other DNA
cttcctctgcctctggtttg

SEQ ID NO: 25 - DNA, 20 bp, synthetic construct
  misc_feature 1..20: note = primer sequence
  source 1..20: mol_type = other DNA
ccatctctgtcctccatgag

SEQ ID NO: 26 - DNA, 20 bp, synthetic construct
  misc_feature 1..20: note = primer sequence
  source 1..20: mol_type = other DNA
atttctgctctgacaacctc

SEQ ID NO: 27 - DNA, 20 bp, synthetic construct
  misc_feature 1..20: note = primer sequence
  source 1..20: mol_type = other DNA
tgcaaaatgggacagaaaga

SEQ ID NO: 28 - DNA, 20 bp, synthetic construct
  misc_feature 1..20: note = primer sequence
  source 1..20: mol_type = other DNA
tgattcagaagcgagtgtgc

SEQ ID NO: 29 - DNA, 20 bp, synthetic construct
  misc_feature 1..20: note = primer sequence
  source 1..20: mol_type = other DNA
accaaatacaggagccatgc

SEQ ID NO: 30 - DNA, 20 bp, synthetic construct
  misc_feature 1..20: note = primer sequence
  source 1..20: mol_type = other DNA
gcgatttccttcttttgcag

SEQ ID NO: 31 - DNA, 20 bp, synthetic construct
  misc_feature 1..20: note = primer sequence
  source 1..20: mol_type = other DNA
cgtctcctaccagaccaagg

SEQ ID NO: 32 - DNA, 20 bp, synthetic construct
  misc_feature 1..20: note = primer sequence
  source 1..20: mol_type = other DNA
ccaaagtagacctgcccaga

SEQ ID NO: 33 - DNA, 20 bp, synthetic construct
  misc_feature 1..20: note = primer sequence
  source 1..20: mol_type = other DNA
tacccccaggagaagattcc

SEQ ID NO: 34 - DNA, 20 bp, synthetic construct
  misc_feature 1..20: note = primer sequence
  source 1..20: mol_type = other DNA
gccatctttggaaggttcag